European Patent Specification EP 3 871 684 B1, published June 26, 2024. Title: Medicament for therapeutic treatment and/or improvement of sepsis. Applicant: Asahi Kasei Pharma Corporation. The sequence listing filed with the application follows.

SEQUENCE LISTING (13 sequences)

SEQ ID NO: 1 - protein, 132 aa, human
MLGVLVLGALALAGLGFPDPCFRANCEYQCQPLNQTSYLCVCAEGFAPIPHEPHRCQMFCNQTACPADCDPNTQASCECPEGYILDDGFICTDIDECENGGFCSGVCHNLPGTFECICGPDSALVRHIGTDC

SEQ ID NO: 2 - DNA, 396 bp, human
atgcttggggtcctggtccttggcgcgctggccctggccggcctggggttccccgacccgtgcttcagagccaactgcgagtaccagtgccagcccctgaaccaaactagctacctctgcgtctgcgccgagggcttcgcgcccattccccacgagccgcacaggtgccagatgttttgcaaccagactgcctgtccagccgactgcgaccccaacacccaggctagctgtgagtgccctgaaggctacatcctggacgacggtttcatctgcacggacatcgacgagtgcgaaaacggcggcttctgctccggggtgtgccacaacctccccggtaccttcgagtgcatctgcgggcccgactcggcccttgtccgccacattggcaccgactgt

SEQ ID NO: 3 - protein, 132 aa, human
MLGVLVLGALALAGLGFPDPCFRANCEYQCQPLNQTSYLCVCAEGFAPIPHEPHRCQMFCNQTACPADCDPNTQASCECPEGYILDDGFICTDIDECENGGFCSGVCHNLPGTFECICGPDSALARHIGTDC

SEQ ID NO: 4 - DNA, 396 bp, human
atgcttggggtcctggtccttggcgcgctggccctggccggcctggggttccccgacccgtgcttcagagccaactgcgagtaccagtgccagcccctgaaccaaactagctacctctgcgtctgcgccgagggcttcgcgcccattccccacgagccgcacaggtgccagatgttttgcaaccagactgcctgtccagccgactgcgaccccaacacccaggctagctgtgagtgccctgaaggctacatcctggacgacggtttcatctgcacggacatcgacgagtgcgaaaacggcggcttctgctccggggtgtgccacaacctccccggtaccttcgagtgcatctgcgggcccgactcggcccttgcccgccacattggcaccgactgt

SEQ ID NO: 5 - protein, 480 aa, human
MLGVLVLGALALAGLGFPAPAEPQPGGSQCVEHDCFALYPGPATFLNASQICDGLRGHLMTVRSSVAADVISLLLNGDGGVGRRRLWIGLQLPPGCGDPKRLGPLRGFQWVTGDNNTSYSRWARLDLNGAPLCGPLCVAVSAAEATVPSEPIWEEQQCEVKADGFLCEFHFPATCRPLAVEPGAAAAAVSITYGTPFAARGADFQALPVGSSAAVAPLGLQLMCTAPPGAVQGHWAREAPGAWDCSVENGGCEHACNAIPGAPRCQCPAGAALQADGRSCTASATQSCNDLCEHFCVPNPDQPGSYSCMCETGYRLAADQHRCEDVDDCILEPSPCPQRCVNTQGGFECHCYPNYDLVDGECVEPVDPCFRANCEYQCQPLNQTSYLCVCAEGFAPIPHEPHRCQMFCNQTACPADCDPNTQASCECPEGYILDDGFICTDIDECENGGFCSGVCHNLPGTFECICGPDSALVRHIGTDC

SEQ ID NO: 6 - DNA, 1440 bp, human
atgcttggggtcctggtccttggcgcgctggccctggccggcctggggttccccgcacccgcagagccgcagccgggtggcagccagtgcgtcgagcacgactgcttcgcgctctacccgggccccgcgaccttcctcaatgccagtcagatctgcgacggactgcggggccacctaatgacagtgcgctcctcggtggctgccgatgtcatttccttgctactgaacggcgacggcggcgttggccgccggcgcctctggatcggcctgcagctgccacccggctgcggcgaccccaagcgcctcgggcccctgcgcggcttccagtgggttacgggagacaacaacaccagctatagcaggtgggcacggctcgacctcaatggggctcccctctgcggcccgttgtgcgtcgctgtctccgctgctgaggccactgtgcccagcgagccgatctgggaggagcagcagtgcgaagtgaaggccgatggcttcctctgcgagttccacttcccagccacctgcaggccactggctgtggagcccggcgccgcggctgccgccgtctcgatcacctacggcaccccgttcgcggcccgcggagcggacttccaggcgctgccggtgggcagctccgccgcggtggctcccctcggcttacagctaatgtgcaccgcgccgcccggagcggtccaggggcactgggccagggaggcgccgggcgcttgggactgcagcgtggagaacggcggctgcgagcacgcgtgcaatgcgatccctggggctccccgctgccagtgcccagccggcgccgccctgcaggcagacgggcgctcctgcaccgcatccgcgacgcagtcctgcaacgacctctgcgagcacttctgcgttcccaaccccgaccagccgggctcctactcgtgcatgtgcgagaccggctaccggctggcggccgaccaacaccggtgcgaggacgtggatgactgcatactggagcccagtccgtgtccgcagcgctgtgtcaacacacagggtggcttcgagtgccactgctaccctaactacgacctggtggacggcgagtgtgtggagcccgtggacccgtgcttcagagccaactgcgagtaccagtgccagcccctgaaccaaactagctacctctgcgtctgcgccgagggcttcgcgcccattccccacgagccgcacaggtgccagatgttttgcaaccagactgcctgtccagccgactgcgaccccaacacccaggctagctgtgagtgccctgaaggctacatcctggacgacggtttcatctgcacggacatcgacgagtgcgaaaacggcggcttctgctccggggtgtgccacaacctccccggtaccttcgagtgcatctgcgggcccgactcggcccttgtccgccacattggcaccgactgt

SEQ ID NO: 7 - protein, 480 aa, human
MLGVLVLGALALAGLGFPAPAEPQPGGSQCVEHDCFALYPGPATFLNASQICDGLRGHLMTVRSSVAADVISLLLNGDGGVGRRRLWIGLQLPPGCGDPKRLGPLRGFQWVTGDNNTSYSRWARLDLNGAPLCGPLCVAVSAAEATVPSEPIWEEQQCEVKADGFLCEFHFPATCRPLAVEPGAAAAAVSITYGTPFAARGADFQALPVGSSAAVAPLGLQLMCTAPPGAVQGHWAREAPGAWDCSVENGGCEHACNAIPGAPRCQCPAGAALQADGRSCTASATQSCNDLCEHFCVPNPDQPGSYSCMCETGYRLAADQHRCEDVDDCILEPSPCPQRCVNTQGGFECHCYPNYDLVDGECVEPVDPCFRANCEYQCQPLNQTSYLCVCAEGFAPIPHEPHRCQMFCNQTACPADCDPNTQASCECPEGYILDDGFICTDIDECENGGFCSGVCHNLPGTFECICGPDSALARHIGTDC

SEQ ID NO: 8 - DNA, 1440 bp, human
atgcttggggtcctggtccttggcgcgctggccctggccggcctggggttccccgcacccgcagagccgcagccgggtggcagccagtgcgtcgagcacgactgcttcgcgctctacccgggccccgcgaccttcctcaatgccagtcagatctgcgacggactgcggggccacctaatgacagtgcgctcctcggtggctgccgatgtcatttccttgctactgaacggcgacggcggcgttggccgccggcgcctctggatcggcctgcagctgccacccggctgcggcgaccccaagcgcctcgggcccctgcgcggcttccagtgggttacgggagacaacaacaccagctatagcaggtgggcacggctcgacctcaatggggctcccctctgcggcccgttgtgcgtcgctgtctccgctgctgaggccactgtgcccagcgagccgatctgggaggagcagcagtgcgaagtgaaggccgatggcttcctctgcgagttccacttcccagccacctgcaggccactggctgtggagcccggcgccgcggctgccgccgtctcgatcacctacggcaccccgttcgcggcccgcggagcggacttccaggcgctgccggtgggcagctccgccgcggtggctcccctcggcttacagctaatgtgcaccgcgccgcccggagcggtccaggggcactgggccagggaggcgccgggcgcttgggactgcagcgtggagaacggcggctgcgagcacgcgtgcaatgcgatccctggggctccccgctgccagtgcccagccggcgccgccctgcaggcagacgggcgctcctgcaccgcatccgcgacgcagtcctgcaacgacctctgcgagcacttctgcgttcccaaccccgaccagccgggctcctactcgtgcatgtgcgagaccggctaccggctggcggccgaccaacaccggtgcgaggacgtggatgactgcatactggagcccagtccgtgtccgcagcgctgtgtcaacacacagggtggcttcgagtgccactgctaccctaactacgacctggtggacggcgagtgtgtggagcccgtggacccgtgcttcagagccaactgcgagtaccagtgccagcccctgaaccaaactagctacctctgcgtctgcgccgagggcttcgcgcccattccccacgagccgcacaggtgccagatgttttgcaaccagactgcctgtccagccgactgcgaccccaacacccaggctagctgtgagtgccctgaaggctacatcctggacgacggtttcatctgcacggacatcgacgagtgcgaaaacggcggcttctgctccggggtgtgccacaacctccccggtaccttcgagtgcatctgcgggcccgactcggcccttgcccgccacattggcaccgactgt

SEQ ID NO: 9 - protein, 516 aa, human
MLGVLVLGALALAGLGFPAPAEPQPGGSQCVEHDCFALYPGPATFLNASQICDGLRGHLMTVRSSVAADVISLLLNGDGGVGRRRLWIGLQLPPGCGDPKRLGPLRGFQWVTGDNNTSYSRWARLDLNGAPLCGPLCVAVSAAEATVPSEPIWEEQQCEVKADGFLCEFHFPATCRPLAVEPGAAAAAVSITYGTPFAARGADFQALPVGSSAAVAPLGLQLMCTAPPGAVQGHWAREAPGAWDCSVENGGCEHACNAIPGAPRCQCPAGAALQADGRSCTASATQSCNDLCEHFCVPNPDQPGSYSCMCETGYRLAADQHRCEDVDDCILEPSPCPQRCVNTQGGFECHCYPNYDLVDGECVEPVDPCFRANCEYQCQPLNQTSYLCVCAEGFAPIPHEPHRCQMFCNQTACPADCDPNTQASCECPEGYILDDGFICTDIDECENGGFCSGVCHNLPGTFECICGPDSALVRHIGTDCDSGKVDGGDSGSGEPPPSPTPGSTLTPPAVGLVHSG

SEQ ID NO: 10 - DNA, 1548 bp, human
atgcttggggtcctggtccttggcgcgctggccctggccggcctggggttccccgcacccgcagagccgcagccgggtggcagccagtgcgtcgagcacgactgcttcgcgctctacccgggccccgcgaccttcctcaatgccagtcagatctgcgacggactgcggggccacctaatgacagtgcgctcctcggtggctgccgatgtcatttccttgctactgaacggcgacggcggcgttggccgccggcgcctctggatcggcctgcagctgccacccggctgcggcgaccccaagcgcctcgggcccctgcgcggcttccagtgggttacgggagacaacaacaccagctatagcaggtgggcacggctcgacctcaatggggctcccctctgcggcccgttgtgcgtcgctgtctccgctgctgaggccactgtgcccagcgagccgatctgggaggagcagcagtgcgaagtgaaggccgatggcttcctctgcgagttccacttcccagccacctgcaggccactggctgtggagcccggcgccgcggctgccgccgtctcgatcacctacggcaccccgttcgcggcccgcggagcggacttccaggcgctgccggtgggcagctccgccgcggtggctcccctcggcttacagctaatgtgcaccgcgccgcccggagcggtccaggggcactgggccagggaggcgccgggcgcttgggactgcagcgtggagaacggcggctgcgagcacgcgtgcaatgcgatccctggggctccccgctgccagtgcccagccggcgccgccctgcaggcagacgggcgctcctgcaccgcatccgcgacgcagtcctgcaacgacctctgcgagcacttctgcgttcccaaccccgaccagccgggctcctactcgtgcatgtgcgagaccggctaccggctggcggccgaccaacaccggtgcgaggacgtggatgactgcatactggagcccagtccgtgtccgcagcgctgtgtcaacacacagggtggcttcgagtgccactgctaccctaactacgacctggtggacggcgagtgtgtggagcccgtggacccgtgcttcagagccaactgcgagtaccagtgccagcccctgaaccaaactagctacctctgcgtctgcgccgagggcttcgcgcccattccccacgagccgcacaggtgccagatgttttgcaaccagactgcctgtccagccgactgcgaccccaacacccaggctagctgtgagtgccctgaaggctacatcctggacgacggtttcatctgcacggacatcgacgagtgcgaaaacggcggcttctgctccggggtgtgccacaacctccccggtaccttcgagtgcatctgcgggcccgactcggcccttgtccgccacattggcaccgactgtgactccggcaaggtggacggtggcgacagcggctctggcgagcccccgcccagcccgacgcccggctccaccttgactcctccggccgtggggctcgtgcattcgggc

SEQ ID NO: 11 - protein, 516 aa, human
MLGVLVLGALALAGLGFPAPAEPQPGGSQCVEHDCFALYPGPATFLNASQICDGLRGHLMTVRSSVAADVISLLLNGDGGVGRRRLWIGLQLPPGCGDPKRLGPLRGFQWVTGDNNTSYSRWARLDLNGAPLCGPLCVAVSAAEATVPSEPIWEEQQCEVKADGFLCEFHFPATCRPLAVEPGAAAAAVSITYGTPFAARGADFQALPVGSSAAVAPLGLQLMCTAPPGAVQGHWAREAPGAWDCSVENGGCEHACNAIPGAPRCQCPAGAALQADGRSCTASATQSCNDLCEHFCVPNPDQPGSYSCMCETGYRLAADQHRCEDVDDCILEPSPCPQRCVNTQGGFECHCYPNYDLVDGECVEPVDPCFRANCEYQCQPLNQTSYLCVCAEGFAPIPHEPHRCQMFCNQTACPADCDPNTQASCECPEGYILDDGFICTDIDECENGGFCSGVCHNLPGTFECICGPDSALARHIGTDCDSGKVDGGDSGSGEPPPSPTPGSTLTPPAVGLVHSG

SEQ ID NO: 12 - DNA, 1548 bp, human
atgcttggggtcctggtccttggcgcgctggccctggccggcctggggttccccgcacccgcagagccgcagccgggtggcagccagtgcgtcgagcacgactgcttcgcgctctacccgggccccgcgaccttcctcaatgccagtcagatctgcgacggactgcggggccacctaatgacagtgcgctcctcggtggctgccgatgtcatttccttgctactgaacggcgacggcggcgttggccgccggcgcctctggatcggcctgcagctgccacccggctgcggcgaccccaagcgcctcgggcccctgcgcggcttccagtgggttacgggagacaacaacaccagctatagcaggtgggcacggctcgacctcaatggggctcccctctgcggcccgttgtgcgtcgctgtctccgctgctgaggccactgtgcccagcgagccgatctgggaggagcagcagtgcgaagtgaaggccgatggcttcctctgcgagttccacttcccagccacctgcaggccactggctgtggagcccggcgccgcggctgccgccgtctcgatcacctacggcaccccgttcgcggcccgcggagcggacttccaggcgctgccggtgggcagctccgccgcggtggctcccctcggcttacagctaatgtgcaccgcgccgcccggagcggtccaggggcactgggccagggaggcgccgggcgcttgggactgcagcgtggagaacggcggctgcgagcacgcgtgcaatgcgatccctggggctccccgctgccagtgcccagccggcgccgccctgcaggcagacgggcgctcctgcaccgcatccgcgacgcagtcctgcaacgacctctgcgagcacttctgcgttcccaaccccgaccagccgggctcctactcgtgcatgtgcgagaccggctaccggctggcggccgaccaacaccggtgcgaggacgtggatgactgcatactggagcccagtccgtgtccgcagcgctgtgtcaacacacagggtggcttcgagtgccactgctaccctaactacgacctggtggacggcgagtgtgtggagcccgtggacccgtgcttcagagccaactgcgagtaccagtgccagcccctgaaccaaactagctacctctgcgtctgcgccgagggcttcgcgcccattccccacgagccgcacaggtgccagatgttttgcaaccagactgcctgtccagccgactgcgaccccaacacccaggctagctgtgagtgccctgaaggctacatcctggacgacggtttcatctgcacggacatcgacgagtgcgaaaacggcggcttctgctccggggtgtgccacaacctccccggtaccttcgagtgcatctgcgggcccgactcggcccttgcccgccacattggcaccgactgtgactccggcaaggtggacggtggcgacagcggctctggcgagcccccgcccagcccgacgcccggctccaccttgactcctccggccgtggggctcgtgcattcgggc

SEQ ID NO: 13 - DNA, 21 bp, Artificial Sequence
  Description of Artificial Sequence: Synthetic DNA
aatgtggcgggcaagggccga